European Patent Application EP 4 596 582 A1, published August 6, 2025. Title: B7-H3 BINDING PROTEIN AND USE THEREOF. Applicant: SICHUAN KELUN-BIOTECH BIOPHARMACEUTICAL CO., LTD. The sequence listing filed with the application follows.

SEQUENCE LISTING (43 sequences)

SEQ ID NO: 1 - protein, 116 aa, synthetic construct
QVQLQESGPGLVKPSGTLSLTCAVSGGSNSSSNWWTWVRQSPGKGLEWIGEISPTGFTSYSPSLKSRVTISVDKSKTQFSLNLSSVTAADTAVYYCARDRLYFDFWGQGTLVTVSS

SEQ ID NO: 2 - protein, 107 aa, synthetic construct
EIVMTQSPATLSVSPGKRATLSCRASQSVSSNLAWYQQKPGQAPRLLIYGASTRATGIPARFSGSGSGTEFTLTISSLQSEDFAVYYCQQYNNWPITFGQGTRLEIK

SEQ ID NO: 3 - protein, 116 aa, synthetic construct
QVQLQESGPGLVQPSGTLSLTCAVSGGSDSSTNWWTWVRQSPGQGLEWIGEISPIGFTSYSPSLRSRVTISVDKSKTQFSLKLSSVTAADTAVYYCARDRLYFAFWGQGTLVTVSS

SEQ ID NO: 4 - protein, 107 aa, synthetic construct
EIVMTQSPATLSVSPGERATLSCRASQSVSSNLAWYQQKPGQAPRLLIYGASTRATGIPDRFSGSGSGTEFTLTISSLESEDFAVYYCQQYNNWPITFGQGTRLEIK

SEQ ID NO: 5 - protein, 9 aa, synthetic construct
GGSNSSSNW

SEQ ID NO: 6 - protein, 7 aa, synthetic construct
ISPTGFT

SEQ ID NO: 7 - protein, 9 aa, synthetic construct
ARDRLYFDF

SEQ ID NO: 8 - protein, 6 aa, synthetic construct
QSVSSN

SEQ ID NO: 9 - skipped

SEQ ID NO: 10 - protein, 9 aa, synthetic construct
QQYNNWPIT

SEQ ID NO: 11 - protein, 8 aa, synthetic construct
GGSNSSSN

SEQ ID NO: 12 - protein, 5 aa, synthetic construct
SPTGF

SEQ ID NO: 13 - protein, 7 aa, synthetic construct
DRLYFDF

SEQ ID NO: 14 - protein, 11 aa, synthetic construct
RASQSVSSNLA

SEQ ID NO: 15 - protein, 7 aa, synthetic construct
GASTRAT

SEQ ID NO: 16 - protein, 6 aa, synthetic construct
SSNWWT

SEQ ID NO: 17 - protein, 16 aa, synthetic construct
EISPTGFTSYSPSLKS

SEQ ID NO: 18 - protein, 9 aa, synthetic construct
GGSDSSTNW

SEQ ID NO: 19 - protein, 7 aa, synthetic construct
ISPIGFT

SEQ ID NO: 20 - protein, 9 aa, synthetic construct
ARDRLYFAF

SEQ ID NO: 21 - protein, 8 aa, synthetic construct
GGSDSSTN

SEQ ID NO: 22 - protein, 5 aa, synthetic construct
SPIGF

SEQ ID NO: 23 - protein, 7 aa, synthetic construct
DRLYFAF

SEQ ID NO: 24 - protein, 6 aa, synthetic construct
STNWWT

SEQ ID NO: 25 - protein, 16 aa, synthetic construct
EISPIGFTSYSPSLRS

SEQ ID NO: 26 - protein, 11 aa, synthetic construct
GGSNSSSNWWT

SEQ ID NO: 27 - protein, 9 aa, synthetic construct
EISPTGFTS

SEQ ID NO: 28 - protein, 11 aa, synthetic construct
GGSDSSTNWWT

SEQ ID NO: 29 - protein, 9 aa, synthetic construct
EISPIGFTS

SEQ ID NO: 30 - protein, 330 aa, synthetic construct [sequence omitted]

SEQ ID NO: 31 - protein, 330 aa, synthetic construct
ASTKGPSVFPLAPSSKSTSGGTAALGCLVKDYFPEPVTVSWNSGALTSGVHTFPAVLQSSGLYSLSSVVTVPSSSLGTQTYICNVNHKPSNTKVDKKVEPKSCDKTHTCPPCPAPEAAGAPSVFLFPPKPKDTLMISRTPEVTCVVVDVSHEDPEVKFNWYVDGVEVHNAKTKPREEQYNSTYRVVSVLTVLHQDWLNGKEYKCKVSNKALPAPIEKTISKAKGQPREPQVYTLPPSRDELTKNQVSLTCLVKGFYPSDIAVEWESNGQPENNYKTTPPVLDSDGSFFLYSKLTVDKSRWQQGNVFSCSVMHEALHNHYTQKSLSLSPGK

SEQ ID NO: 32 - protein, 107 aa, synthetic construct [sequence omitted]

SEQ ID NO: 33 - DNA, 348 bp, synthetic construct
  source 1..348: mol_type = other DNA
caggttcaattgcaagaaagcggccccgggctggtaaaaccaagtggcaccctgagcctgacgtgtgctgtgtctggggggagcaattcctcaagcaattggtggacatgggtgaggcagtcccccggaaagggcttggaatggatcggcgagatcagccctacaggttttaccagctactcccctagcctgaaatccagggtgacgatcagtgtcgacaagtctaaaacacagttctctctgaacctttcaagtgtcactgcagccgatactgctgtgtattactgcgccagagatcggctgtattttgacttttggggccagggcactctggtcacagtgtctagc

SEQ ID NO: 34 - DNA, 321 bp, synthetic construct
  source 1..321: mol_type = other DNA
gaaatagtgatgacccaatcccccgcaactctgtctgtgtcccctgggaagagagccaccctttcctgtcgcgcctcacaatccgtgagctcaaatctggcatggtatcaacagaaaccaggccaagcgcctcggctgctgatttacggcgcctctacccgcgctaccggaatcccagcacgctttagcggctcagggtccggcactgagttcaccttgacaattagtagtctgcagtccgaagattttgccgtctattactgccagcagtataataactggccaatcacctttggccagggcacacgcctggagatcaag

SEQ ID NO: 35 - DNA, 348 bp, synthetic construct
  source 1..348: mol_type = other DNA
caagtacaactccaagaaagtgggccaggactcgtgcaaccatctggcaccctctctctcacctgcgcagtgtctggcggctccgattcttccaccaactggtggacctgggtgagacagtccccaggccaaggattggaatggattggcgagatttcccctattgggttcaccagctacagccccagcctgaggagcagggtgactatcagcgtggataagtctaaaacccagttcagtctcaaactgagtagtgtgactgccgcggacacggcagtgtattattgcgcccgggaccgcctttatttcgccttctgggggcagggcactttggtgaccgtcagtagc

SEQ ID NO: 36 - DNA, 321 bp, synthetic construct
  source 1..321: mol_type = other DNA
gagattgtcatgacacagagtcctgctaccttgtcagttagtcctggggagagagcaacactgtcctgccgcgctagccaaagtgttagctccaacctggcctggtaccagcagaaacccgggcaggcacccagactcctgatttacggagcctctacacgcgcaactggaatccctgaccggttctcaggatccgggagtggcacggaattcaccttgaccattagcagcctggaatccgaagattttgcagtgtattactgtcagcagtacaacaactggcctatcacgttcgggcaggggaccagattggaaatcaag

SEQ ID NO: 37 - DNA, 990 bp, synthetic construct
  source 1..990: mol_type = other DNA
gcatctactaaaggcccaagtgtttttcctctggccccatcctcaaaaagcacctccggaggcacagctgcgctgggatgcctcgtgaaagattatttccctgaacctgttaccgtgtcatggaacagcggcgctctcacttctggcgtgcacacatttcccgctgtgttgcagtccagcggactctatagcctgagctccgtggttacagtgccctcttcatctttgggcacccagacctacatatgcaatgtgaatcataaaccgagcaataccaaggtagataaaaaggtagagccaaaaagttgcgataagactcatacatgcccaccttgtcctgccccggagctgctcggaggaccaagcgtgtttctcttcccccccaagccaaaggataccttgatgattagtcgcaccccagaagtgacatgcgtggtggttgacgtcagccacgaggacccagaggtgaagtttaattggtacgtggacggtgtggaagtccacaatgcaaaaaccaagcctcgcgaagaacagtataacagtacctacagggtcgtcagtgtcctgaccgtgctgcaccaggactggctcaatggaaaggaatacaagtgtaaggtctccaacaaggccttgccagctcccattgaaaagaccattagcaaggccaaaggtcagcctcgcgaaccacaagtgtacacactgcctccgtcacgcgatgaacttaccaaaaatcaggtatcactgacctgccttgtaaagggcttttacccgagtgacatagcagtcgagtgggaatccaacggtcagccggagaacaactataaaaccactcccccagtgcttgattccgatggcagcttcttcctgtacagtaaactgactgtggataagtctcgctggcagcagggcaatgtgttttcttgctctgtcatgcacgaggcacttcacaaccactacacacagaaaagtctcagtctgagtccagggaaa

SEQ ID NO: 38 - DNA, 321 bp, synthetic construct
  source 1..321: mol_type = other DNA
agaacagtggccgcaccaagcgtgtttatctttcctccctctgacgaacaattgaagagtgggaccgcctcagtggtgtgtctgctgaacaatttctacccccgggaggcaaaggtgcagtggaaggtggataatgcactccagtccgggaatagtcaggaaagcgtgactgagcaagacagcaaagactctacatattctctgtccagtaccctgaccctcagcaaggctgattatgagaagcacaaggtgtacgcctgtgaggtcactcaccagggactgagttcaccggtcactaaaagctttaacagaggagagtgc

SEQ ID NO: 39 - DNA, 990 bp, synthetic construct
  source 1..990: mol_type = other DNA
gcctctacaaaaggaccatcagtctttccattggctccgagtagcaaaagcaccagcggtggaacagctgctctggggtgcctggtcaaggactatttccccgagcctgtgaccgtctcttggaacagcggggcactgacctccggtgtccatacatttcctgcagtgctgcaaagttctggattgtattcactctcctctgtcgtgacggttcctagttcatccctgggcacccagacttatatttgcaatgtcaaccacaaacccagcaatactaaagtggataagaaggtcgaacccaagtcttgcgataagacacacacatgccctccttgtcccgcaccagaggctgctggagcaccatcagtgtttcttttcccacctaagcccaaggatacactgatgattagtcgcacacccgaagtgacatgcgtcgtcgtagacgtgagccacgaggaccctgaggtgaaatttaactggtacgtggatggagtggaggtacataatgcaaagacaaaaccccgagaagagcagtacaacagcacttacagggtggtgtccgttctgacagtcctgcatcaggattggcttaacggtaaagaatataagtgtaaagttagtaataaggccctgcccgcccccattgagaagactattagtaaggccaagggacagcccagggaacctcaggtgtataccctgccaccctcccgggacgaactgacaaaaaatcaggtatcattgacctgcctcgtgaagggcttttatccctcagatatagccgtggaatgggagtcaaatggccagcctgagaacaattacaagactacgcctcccgtgctggattctgatggatcattttttctgtacagcaagctgaccgtggataagtcccggtggcagcaggggaacgtgttctcttgctccgtgatgcacgaggcacttcataaccattatacccaaaagtctctctcactgtcccccggcaaa

SEQ ID NO: 40 - protein, 446 aa, synthetic construct
QVQLQESGPGLVKPSGTLSLTCAVSGGSNSSSNWWTWVRQSPGKGLEWIGEISPTGFTSYSPSLKSRVTISVDKSKTQFSLNLSSVTAADTAVYYCARDRLYFDFWGQGTLVTVSSASTKGPSVFPLAPSSKSTSGGTAALGCLVKDYFPEPVTVSWNSGALTSGVHTFPAVLQSSGLYSLSSVVTVPSSSLGTQTYICNVNHKPSNTKVDKKVEPKSCDKTHTCPPCPAPELLGGPSVFLFPPKPKDTLMISRTPEVTCVVVDVSHEDPEVKFNWYVDGVEVHNAKTKPREEQYNSTYRVVSVLTVLHQDWLNGKEYKCKVSNKALPAPIEKTISKAKGQPREPQVYTLPPSRDELTKNQVSLTCLVKGFYPSDIAVEWESNGQPENNYKTTPPVLDSDGSFFLYSKLTVDKSRWQQGNVFSCSVMHEALHNHYTQKSLSLSPGK

SEQ ID NO: 41 - protein, 214 aa, synthetic construct
EIVMTQSPATLSVSPGKRATLSCRASQSVSSNLAWYQQKPGQAPRLLIYGASTRATGIPARFSGSGSGTEFTLTISSLQSEDFAVYYCQQYNNWPITFGQGTRLEIKRTVAAPSVFIFPPSDEQLKSGTASVVCLLNNFYPREAKVQWKVDNALQSGNSQESVTEQDSKDSTYSLSSTLTLSKADYEKHKVYACEVTHQGLSSPVTKSFNRGEC

SEQ ID NO: 42 - protein, 446 aa, synthetic construct
QVQLQESGPGLVQPSGTLSLTCAVSGGSDSSTNWWTWVRQSPGQGLEWIGEISPIGFTSYSPSLRSRVTISVDKSKTQFSLKLSSVTAADTAVYYCARDRLYFAFWGQGTLVTVSSASTKGPSVFPLAPSSKSTSGGTAALGCLVKDYFPEPVTVSWNSGALTSGVHTFPAVLQSSGLYSLSSVVTVPSSSLGTQTYICNVNHKPSNTKVDKKVEPKSCDKTHTCPPCPAPEAAGAPSVFLFPPKPKDTLMISRTPEVTCVVVDVSHEDPEVKFNWYVDGVEVHNAKTKPREEQYNSTYRVVSVLTVLHQDWLNGKEYKCKVSNKALPAPIEKTISKAKGQPREPQVYTLPPSRDELTKNQVSLTCLVKGFYPSDIAVEWESNGQPENNYKTTPPVLDSDGSFFLYSKLTVDKSRWQQGNVFSCSVMHEALHNHYTQKSLSLSPGK

SEQ ID NO: 43 - protein, 214 aa, synthetic construct
EIVMTQSPATLSVSPGERATLSCRASQSVSSNLAWYQQKPGQAPRLLIYGASTRATGIPDRFSGSGSGTEFTLTISSLESEDFAVYYCQQYNNWPITFGQGTRLEIKRTVAAPSVFIFPPSDEQLKSGTASVVCLLNNFYPREAKVQWKVDNALQSGNSQESVTEQDSKDSTYSLSSTLTLSKADYEKHKVYACEVTHQGLSSPVTKSFNRGEC